European Patent Application EP 4 686 758 A1, published February 4, 2026. Title: NUCLEIC ACID FOR NUCLEAR TRANSLOCATION. Applicant: 4basebio UK Ltd. Application EP. The sequence listing filed with the application follows.

SEQUENCE LISTING (28 sequences)

SEQ ID NO: 1 - protein, 6 aa, synthetic construct
PKLKRQ

SEQ ID NO: 2 - protein, 4 aa, synthetic construct
RPRK

SEQ ID NO: 3 - protein, 8 aa, synthetic construct
RRARRPRG

SEQ ID NO: 4 - protein, 21 aa, synthetic construct
GKRKLITSEEERSPAKRGRKS

SEQ ID NO: 5 - protein, 22 aa, synthetic construct
KGKKGRTQKEKKAARARSKGKN

SEQ ID NO: 6 - protein, 28 aa, synthetic construct
RKRCAAGVGGGPAGCPAPGSTPLKKPRR

SEQ ID NO: 7 - protein, 36 aa, synthetic construct
RKPVTAQERQREREEKRRRRQERAKEREKRRQERER

SEQ ID NO: 8 - protein, 27 aa, synthetic construct
RSGGNHRRNGRGGRGGYNRRNNGYHPY

SEQ ID NO: 9 - protein, 27 aa, synthetic construct
TLLLRETMNNLGVSDHAVLSRKTPQPY

SEQ ID NO: 10 - protein, 18 aa, synthetic construct
PGKMDKGEHRQERRDRPY

SEQ ID NO: 11 - protein, 21 aa, synthetic construct
GKKKKGKPGKRREQRKKKRRT

SEQ ID NO: 12 - protein, 27 aa, synthetic construct
SANKVTKNKSNSSPYLNKRKGKPGPDS

SEQ ID NO: 13 - protein, 43 aa, synthetic construct
VHSHKKKKIPTSPTFTTPKTLTLRRQPKYPRKSAPRRNKLDHY

SEQ ID NO: 14 - protein, 10 aa, synthetic construct
RKHKTNRKPR

SEQ ID NO: 15 - protein, 8 aa, synthetic construct
NRRAKAKR

SEQ ID NO: 16 - protein, 6 aa, synthetic construct
RNKKKK

SEQ ID NO: 17 - protein, 5 aa, synthetic construct
RKVIK

SEQ ID NO: 18 - protein, 7 aa, synthetic construct
PKKKRKV

SEQ ID NO: 19 - protein, 9 aa, synthetic construct
PAAKRVKLD

SEQ ID NO: 20 - protein, 16 aa, synthetic construct
KRPAATKKAGQAKKKK

SEQ ID NO: 21 - protein, 16 aa, synthetic construct
TRQARRNRRRRWRERQ

SEQ ID NO: 22 - protein, 12 aa, synthetic construct
PKKKRKVEDPYC

SEQ ID NO: 23 - DNA, 55 bp, synthetic construct
  source 1..55: mol_type = other DNA
ggggactttccggggactttccggggactttccggggactttccggggactttcc

SEQ ID NO: 24 - DNA, 144 bp, synthetic construct
  source 1..144: mol_type = other DNA
tggttgctgactaattgagatgcatgctttgcatacttctgcctgctggggagcctggggactttccacacctggttgctgactaattgagatgcatgctttgcatacttctgcctgctggggagcctggggactttccacacc

SEQ ID NO: 25 - DNA, 16 bp, synthetic construct
  source 1..16: mol_type = other DNA
  modified_base 1..5: mod_base = OTHER; note = phosphorothioated nucleotide
ggccaacaaatgttag

SEQ ID NO: 26 - DNA, 20 bp, synthetic construct
  source 1..20: mol_type = other DNA
  modified_base 16..20: mod_base = OTHER; note = phosphorothioated nucleotide
agggctaacatttgttggcc

SEQ ID NO: 27 - DNA, 120 bp, synthetic construct
  misc_feature 1..14: note = DNA
  misc_feature 111..120: note = DNA
  source 1..120: mol_type = other DNA
  misc_feature 15..110: note = RNA
agggctaacatttggatcctgagctactgactttgggtcgaattggttggctcgccctcttcttggaattcaggagggcgattgaacggacaccactactgaccatacaccaaatgttag

SEQ ID NO: 28 - protein, 22 aa, synthetic construct
CGKRKLITSEEERSPAKRGRKS